European Patent Application EP 4 733 418 A1, published April 29, 2026. Title: METHOD FOR TAXONOMIC AND STRAIN TYPE IDENTIFICATION OF BACTERIA AND ARCHAEA. Applicant: Marco MEOLA. Application EP. The sequence listing filed with the application follows.

SEQUENCE LISTING (3 sequences)

SEQ ID NO: 1 - DNA, 20 bp, synthetic construct
  source 1..20: mol_type = other DNA
  unsure 7
gttcggnatggrwhsrggyg

SEQ ID NO: 2 - DNA, 20 bp, synthetic construct
  source 1..20: mol_type = other DNA
  unsure 7
gttcgrnawggddhsrsgyg

SEQ ID NO: 3 - DNA, 20 bp, synthetic construct
  source 1..20: mol_type = other DNA
agrrttygatyhtdgytyag